European Patent Application EP 4 292 664 A2, published December 20, 2023. Title: ANTAGONISTIC ANTI-TUMOR NECROSIS FACTOR RECEPTOR SUPERFAMILY ANTIBODIES. Applicant: THE GENERAL HOSPITAL CORPORATION. Application AU 2023200440, filed January 27, 2023. The sequence listing filed with the application follows.

SEQUENCE LISTING (283 sequences)

SEQ ID NO: 1 - DNA, 523 bp, Mus sp.
  source 1..523: mol_type = genomic DNA
gaccaggcatcccagggtcaccatggagttagtttgggcagcagatccaggggccagtggatagacagatgggggtgtcgttttggctgaggagacggtgaccgcggtccctgcgccccagacatcgaagtaccagtagctggagtaaccatcaaccctctgtcgtgcacagtaatacatggccgtgtcctcagacctcagactgctcatttgcaggtacagggtgttcttggcattgtctctggagatggtgaatcgccccttcacactgtctggatagtaggtgtaactaccaccactactaatggttgcgacccactccagcctcttctccggagtctggcgaacccaagacatgacataactactgaaagtgaatccagaggctgcacaggagagtttcagggaccctccaggcttcactaagcctccccctgactcctgcagctgcacctccggaagcctgaattctgcagatatccatcacactggcggccgctcgagcatgcatctagaggcccat

SEQ ID NO: 2 - protein, 123 aa, Mus sp.
EVQLQESGGGLVKPGGSLKLSCAASGFTFSSYVMSWVRQTPEKRLEWVATISSGGSYTYYPDSVKGRFTISRDNAKNTLYLQMSSLRSEDTAMYYCARQRVDGYSSYWYFDVWGAGTAVTVSS

SEQ ID NO: 3 - DNA, 508 bp, Mus sp.
  source 1..508: mol_type = genomic DNA
ctccgagcggccgccagtgtgatggatatctgcagaattcagggggacattgtgctgacccagtctccagcaatcatgtctgcatctccaggggagaaggtcaccataacctgcagtgccagctcaagtgtatattacatgtactggttccagcagaagccaggcacttctcccaaactctggatttatagcacatccaacctggcttctggagtccctgttcgcttcagtggcagtggctctgggacctcttactctctcacaatcagccgaatggaggctgaagatgctgccacttattactgccagcaaaggaggaattacccgtacacgttcggaggggggaccaagttggaaataaaacgggctgatgctccaccaactgtatccatcttcccaccatccagtgagcagttacctgaattccagcacactggcggccgttactagtggatccgagctcggtaccaagcttgatgcatagcttgagtattctaacgcgtcacct

SEQ ID NO: 4 - protein, 108 aa, Mus sp.
DIVLTQSPAIMSASPGEKVTITCSASSSVYYMYWFQQKPGTSPKLWIYSTSNLASGVPVRFSGSGSGTSYSLTISRMEAEDAATYYCQQRRNYPYTFGGGTKLEIKRA

SEQ ID NO: 5 - DNA, 454 bp, Mus sp.
  source 1..454: mol_type = genomic DNA
gagcggccgccagtgtgatggatatctgcagaattcagggggacattgtgctgacccagactcctgcttccttagctgtatctctggggcagagggccaccatctcatgcagggccagcaaaagtgtcagtacatctggctatagttatatgcactggtaccaacagaaaccaggacagccacccaaactcctcatctatcttgcatccaacctagaatctggggtccctgccaggttcagtggcagtgggtctgggacagacttcaccctcaacatccatcctgtggaggaggaggatgctgcaacctattactgtcagcacagtagggagcttcctcggacgttcggtggaggcaccaagctggaaatcaaacgggctgatgctccaccaactgtatccacccctgaattccagcacactggcggccgttactagtggatccgagctcggta

SEQ ID NO: 6 - protein, 113 aa, Mus sp.
DIVLTQTPASLAVSLGQRATISCRASKSVSTSGYSYMHWYQQKPGQPPKLLIYLASNLESGVPARFSGSGSGTDFTLNIHPVEEEDAATYYCQHSRELPRTFGGGTKLEIKRA

SEQ ID NO: 7 - protein, 461 aa, Homo sapiens
MAPVAVWAALAVGLELWAAAHALPAQVAFTPYAPEPGSTCRLREYYDQTAQMCCSKCSPGQHAKVFCTKTSDTVCDSCEDSTYTQLWNWVPECLSCGSRCSSDQVETQACTREQNRICTCRPGWYCALSKQEGCRLCAPLRKCRPGFGVARPGTETSDVVCKPCAPGTFSNTTSSTDICRPHQICNVVAIPGNASMDAVCTSTSPTRSMAPGAVHLPQPVSTRSQHTQPTPEPSTAPSTSFLLPMGPSPPAEGSTGDFALPVGLIVGVTALGLLIIGVVNCVIMTQVKKKPLCLQREAKVPHLPADKARGTQGPEQQHLLITAPSSSSSSLESSASALDRRAPTRNQPQAPGVEASGAGEARASTGSSDSSPGGHGTQVNVTCIVNVCSSSDHSSQCSSQASSTMGDTDSSPSESPKDEQVPFSKEECAFRSQLETPETLLGSTEEKPLPLGVPDAGMKPS

SEQ ID NO: 8 - protein, 7 aa, Homo sapiens
DSTYTQL

SEQ ID NO: 9 - protein, 8 aa, Homo sapiens
PECLSCGS

SEQ ID NO: 10 - protein, 8 aa, Homo sapiens
RICTCRPG

SEQ ID NO: 11 - protein, 8 aa, Homo sapiens
CAPLRKCR

SEQ ID NO: 12 - protein, 5 aa, Homo sapiens
KCSPG

SEQ ID NO: 13 - protein, 54 aa, Homo sapiens
CDSCEDSTYTQLWNWVPECLSCGSRCSSDQVETQACTREQNRICTCRPGWYCAL

SEQ ID NO: 14 - protein, 17 aa, Homo sapiens
CDSCEDSTYTQLWNWVP

SEQ ID NO: 15 - protein, 18 aa, Homo sapiens
LWNWVPECLSCGSRCSSD

SEQ ID NO: 16 - protein, 18 aa, Homo sapiens
TREQNRICTCRPGWYCAL

SEQ ID NO: 17 - protein, 20 aa, Homo sapiens
KQEGCRLCAPLRKCRPGFGV

SEQ ID NO: 18 - protein, 20 aa, Homo sapiens
QTAQMCCSKCSPGQHAKVFC

SEQ ID NO: 19 - protein, 5 aa, Homo sapiens
KCRPG

SEQ ID NO: 20 - protein, 8 aa, Homo sapiens
KCRPGFGV

SEQ ID NO: 21 - protein, 9 aa, Homo sapiens
CKPCAPGTF

SEQ ID NO: 22 - protein, 41 aa, Homo sapiens
ARPGTETSDVVCKPCAPGTFSNTTSSTDICRPHQICNVVAI

SEQ ID NO: 23 - protein, 7 aa, Mus sp.
GFTFSSY

SEQ ID NO: 24 - protein, 6 aa, Mus sp.
SSGGSY

SEQ ID NO: 25 - protein, 14 aa, Mus sp.
QRVDGYSSYWYFDV

SEQ ID NO: 26 - protein, 10 aa, Mus sp.
SASSSVYYMY

SEQ ID NO: 27 - protein, 7 aa, Mus sp.
STSNLAS

SEQ ID NO: 28 - protein, 9 aa, Mus sp.
QQRRNYPYT

SEQ ID NO: 29 - protein, 15 aa, Mus sp.
RASKSVSTSGYSYMH

SEQ ID NO: 30 - protein, 7 aa, Mus sp.
LASNLES

SEQ ID NO: 31 - protein, 9 aa, Mus sp.
QHSRELPRT

SEQ ID NO: 32 - protein, 120 aa, Homo sapiens
EVQLVESGGGLVQPGGSLRLSCAASGFTFSDYAMSWVRQAPGKGLEWVAVISENGSDTYYADSVKGRFTISRDDSKNTLYLQMNSLRAEDTAVYYCARDRGGAVSYFDVWGQGTLVTVSS

SEQ ID NO: 33 - protein, 109 aa, Homo sapiens
DIQMTQSPSSLSASVGDRVTITCRASQDVSSYLAWYQQKPGKAPKLLIYAASSLESGVPSRFSGSGSGTDFTLTISSLQPEDFATYYCQQYNSLPYTFGQGTKVEIKRT

SEQ ID NO: 34 - protein, 27 aa, synthetic construct
  SITE 3: note = Cys residue protected with ACM protecting group
  SITE 6: note = Cys residue protected with ACM protecting group
  SITE 22: note = Cys residue protected with ACM protecting group
PECLSCGSRCSGGSGGNRICTCRPGWY

SEQ ID NO: 35 - protein, 27 aa, synthetic construct
  SITE 1: note = Cys residue protected with ACM protecting group
  SITE 4: note = Cys residue protected with ACM protecting group
  SITE 22: note = Cys residue protected with ACM protecting group
CLSCGSRCSSDGGSGGNRICTCRPGWY

SEQ ID NO: 36 - protein, 27 aa, synthetic construct
  SITE 4: note = Cys residue protected with ACM protecting group
  SITE 7: note = Cys residue protected with ACM protecting group
  SITE 22: note = Cys residue protected with ACM protecting group
VPECLSCGSRCGGSGGNRICTCRPGWY

SEQ ID NO: 37 - protein, 27 aa, synthetic construct
  SITE 3: note = Cys residue protected with ACM protecting group
  SITE 22: note = Cys residue protected with ACM protecting group
LSCGSRCSSDQGGSGGNRICTCRPGWY

SEQ ID NO: 38 - protein, 27 aa, synthetic construct
  SITE 3: note = Cys residue protected with ACM protecting group
  SITE 6: note = Cys residue protected with ACM protecting group
  SITE 19: note = Cys residue protected with ACM protecting group
  SITE 25: note = Cys residue protected with ACM protecting group
PECLSCGSRCSGGSGGCTCRPGWYCAL

SEQ ID NO: 39 - protein, 27 aa, synthetic construct
  SITE 2: note = Cys residue protected with ACM protecting group
  SITE 22: note = Cys residue protected with ACM protecting group
SCGSRCSSDQVGGSGGNRICTCRPGWY

SEQ ID NO: 40 - protein, 27 aa, synthetic construct
  SITE 1: note = Cys residue protected with ACM protecting group
  SITE 21: note = Cys residue protected with ACM protecting group
  SITE 27: note = Cys residue protected with ACM protecting group
CGSRCSSDQVEGGSGGRICTCRPGWYC

SEQ ID NO: 41 - protein, 27 aa, synthetic construct
  SITE 2: note = Cys residue protected with ACM protecting group
  SITE 5: note = Cys residue protected with ACM protecting group
  SITE 19: note = Cys residue protected with ACM protecting group
  SITE 25: note = Cys residue protected with ACM protecting group
ECLSCGSRCSSGGSGGCTCRPGWYCAL

SEQ ID NO: 42 - protein, 27 aa, synthetic construct
  SITE 6: note = Cys residue protected with ACM protecting group
  SITE 17: note = Cys residue protected with ACM protecting group
EGCRLCAPLRKGGSGGCAPLRKCRPGF

SEQ ID NO: 43 - protein, 27 aa, synthetic construct
  SITE 1: note = Cys residue protected with ACM protecting group
  SITE 4: note = Cys residue protected with ACM protecting group
  SITE 19: note = Cys residue protected with ACM protecting group
  SITE 25: note = Cys residue protected with ACM protecting group
CLSCGSRCSSDGGSGGCTCRPGWYCAL

SEQ ID NO: 44 - protein, 27 aa, synthetic construct
  SITE 11: note = Cys residue protected with ACM protecting group
  SITE 21: note = Cys residue protected with ACM protecting group
  SITE 27: note = Cys residue protected with ACM protecting group
CSSDQVETQACGGSGGRICTCRPGWYC

SEQ ID NO: 45 - protein, 27 aa, synthetic construct
  SITE 21: note = Cys residue protected with ACM protecting group
  SITE 27: note = Cys residue protected with ACM protecting group
GSRCSSDQVETGGSGGRICTCRPGWYC

SEQ ID NO: 46 - protein, 27 aa, synthetic construct
  SITE 1: note = Cys residue protected with ACM protecting group
  SITE 22: note = Cys residue protected with ACM protecting group
CGSRCSSDQVEGGSGGNRICTCRPGWY

SEQ ID NO: 47 - protein, 27 aa, synthetic construct
  SITE 22: note = Cys residue protected with ACM protecting group
GSRCSSDQVETGGSGGNRICTCRPGWY

SEQ ID NO: 48 - protein, 27 aa, synthetic construct
  SITE 3: note = Cys residue protected with ACM protecting group
  SITE 6: note = Cys residue protected with ACM protecting group
  SITE 21: note = Cys residue protected with ACM protecting group
  SITE 27: note = Cys residue protected with ACM protecting group
PECLSCGSRCSGGSGGRICTCRPGWYC

SEQ ID NO: 49 - protein, 27 aa, synthetic construct
  SITE 4: note = Cys residue protected with ACM protecting group
  SITE 7: note = Cys residue protected with ACM protecting group
  SITE 23: note = Cys residue protected with ACM protecting group
VPECLSCGSRCGGSGGQNRICTCRPGW

SEQ ID NO: 50 - protein, 27 aa, synthetic construct
  SITE 7: note = Cys residue protected with ACM protecting group
  SITE 17: note = Cys residue protected with ACM protecting group
QEGCRLCAPLRGGSGGCAPLRKCRPGF

SEQ ID NO: 51 - protein, 27 aa, synthetic construct
  SITE 21: note = Cys residue protected with ACM protecting group
  SITE 27: note = Cys residue protected with ACM protecting group
SRCSSDQVETQGGSGGRICTCRPGWYC

SEQ ID NO: 52 - protein, 27 aa, synthetic construct
  SITE 11: note = Cys residue protected with ACM protecting group
  SITE 17: note = Cys residue protected with ACM protecting group
ALSKQEGCRLCGGSGGCAPLRKCRPGF

SEQ ID NO: 53 - protein, 27 aa, synthetic construct
  SITE 7: note = Cys residue protected with ACM protecting group
QEGCRLCAPLRGGSGGPLRKCRPGFGV

SEQ ID NO: 54 - protein, 27 aa, synthetic construct
  SITE 2: note = Cys residue protected with ACM protecting group
YCALSKQEGCRGGSGGAPLRKCRPGFG

SEQ ID NO: 55 - protein, 27 aa, synthetic construct
  SITE 3: note = Cys residue protected with ACM protecting group
  SITE 21: note = Cys residue protected with ACM protecting group
  SITE 27: note = Cys residue protected with ACM protecting group
LSCGSRCSSDQGGSGGRICTCRPGWYC

SEQ ID NO: 56 - protein, 27 aa, synthetic construct
  SITE 3: note = Cys residue protected with ACM protecting group
  SITE 6: note = Cys residue protected with ACM protecting group
  SITE 23: note = Cys residue protected with ACM protecting group
PECLSCGSRCSGGSGGQNRICTCRPGW

SEQ ID NO: 57 - protein, 27 aa, synthetic construct
  SITE 21: note = Cys residue protected with ACM protecting group
  SITE 27: note = Cys residue protected with ACM protecting group
RCSSDQVETQAGGSGGRICTCRPGWYC

SEQ ID NO: 58 - protein, 27 aa, synthetic construct
  SITE 3: note = Cys residue protected with ACM protecting group
  SITE 6: note = Cys residue protected with ACM protecting group
  SITE 20: note = Cys residue protected with ACM protecting group
  SITE 26: note = Cys residue protected with ACM protecting group
PECLSCGSRCSGGSGGICTCRPGWYCA

SEQ ID NO: 59 - protein, 27 aa, synthetic construct
  SITE 4: note = Cys residue protected with ACM protecting group
  SITE 7: note = Cys residue protected with ACM protecting group
  SITE 20: note = Cys residue protected with ACM protecting group
  SITE 26: note = Cys residue protected with ACM protecting group
VPECLSCGSRCGGSGGICTCRPGWYCA

SEQ ID NO: 60 - protein, 27 aa, synthetic construct
  SITE 2: note = Cys residue protected with ACM protecting group
  SITE 19: note = Cys residue protected with ACM protecting group
  SITE 25: note = Cys residue protected with ACM protecting group
SCGSRCSSDQVGGSGGCTCRPGWYCAL

SEQ ID NO: 61 - protein, 27 aa, synthetic construct
  SITE 3: note = Cys residue protected with ACM protecting group
WYCALSKQEGCGGSGGAPLRKCRPGFG

SEQ ID NO: 62 - protein, 27 aa, synthetic construct
  SITE 10: note = Cys residue protected with ACM protecting group
  SITE 17: note = Cys residue protected with ACM protecting group
LSKQEGCRLCAGGSGGCAPLRKCRPGF

SEQ ID NO: 63 - protein, 27 aa, synthetic construct
  SITE 8: note = Cys residue protected with ACM protecting group
  SITE 17: note = Cys residue protected with ACM protecting group
KQEGCRLCAPLGGSGGCAPLRKCRPGF

SEQ ID NO: 64 - protein, 27 aa, synthetic construct
  SITE 3: note = Cys residue protected with ACM protecting group
  SITE 19: note = Cys residue protected with ACM protecting group
  SITE 25: note = Cys residue protected with ACM protecting group
LSCGSRCSSDQGGSGGCTCRPGWYCAL

SEQ ID NO: 65 - protein, 27 aa, synthetic construct
  SITE 23: note = Cys residue protected with ACM protecting group
RCSSDQVETQAGGSGGQNRICTCRPGW

SEQ ID NO: 66 - protein, 27 aa, synthetic construct
  SITE 9: note = Cys residue protected with ACM protecting group
  SITE 17: note = Cys residue protected with ACM protecting group
SKQEGCRLCAPGGSGGCAPLRKCRPGF

SEQ ID NO: 67 - protein, 27 aa, synthetic construct
  SITE 1: note = Cys residue protected with ACM protecting group
  SITE 23: note = Cys residue protected with ACM protecting group
CGSRCSSDQVEGGSGGQNRICTCRPGW

SEQ ID NO: 68 - protein, 27 aa, synthetic construct
  SITE 11: note = Cys residue protected with ACM protecting group
  SITE 23: note = Cys residue protected with ACM protecting group
CSSDQVETQACGGSGGQNRICTCRPGW

SEQ ID NO: 69 - protein, 27 aa, synthetic construct
  SITE 11: note = Cys residue protected with ACM protecting group
  SITE 22: note = Cys residue protected with ACM protecting group
CSSDQVETQACGGSGGNRICTCRPGWY

SEQ ID NO: 70 - protein, 27 aa, synthetic construct
  SITE 4: note = Cys residue protected with ACM protecting group
  SITE 7: note = Cys residue protected with ACM protecting group
  SITE 19: note = Cys residue protected with ACM protecting group
  SITE 25: note = Cys residue protected with ACM protecting group
VPECLSCGSRCGGSGGCTCRPGWYCAL

SEQ ID NO: 71 - protein, 27 aa, synthetic construct
  SITE 2: note = Cys residue protected with ACM protecting group
  SITE 5: note = Cys residue protected with ACM protecting group
  SITE 23: note = Cys residue protected with ACM protecting group
ECLSCGSRCSSGGSGGQNRICTCRPGW

SEQ ID NO: 72 - protein, 27 aa, synthetic construct
  SITE 22: note = Cys residue protected with ACM protecting group
SRCSSDQVETQGGSGGNRICTCRPGWY

SEQ ID NO: 73 - protein, 27 aa, synthetic construct
  SITE 1: note = Cys residue protected with ACM protecting group
  SITE 19: note = Cys residue protected with ACM protecting group
  SITE 25: note = Cys residue protected with ACM protecting group
CGSRCSSDQVEGGSGGCTCRPGWYCAL

SEQ ID NO: 74 - protein, 27 aa, synthetic construct
  SITE 4: note = Cys residue protected with ACM protecting group
  SITE 7: note = Cys residue protected with ACM protecting group
  SITE 21: note = Cys residue protected with ACM protecting group
  SITE 27: note = Cys residue protected with ACM protecting group
VPECLSCGSRCGGSGGRICTCRPGWYC

SEQ ID NO: 75 - protein, 27 aa, synthetic construct
  SITE 2: note = Cys residue protected with ACM protecting group
  SITE 5: note = Cys residue protected with ACM protecting group
  SITE 21: note = Cys residue protected with ACM protecting group
  SITE 27: note = Cys residue protected with ACM protecting group
ECLSCGSRCSSGGSGGRICTCRPGWYC

SEQ ID NO: 76 - protein, 27 aa, synthetic construct
  SITE 10: note = Cys residue protected with ACM protecting group
LSKQEGCRLCAGGSGGRKCRPGFGVAR

SEQ ID NO: 77 - protein, 27 aa, synthetic construct
  SITE 23: note = Cys residue protected with ACM protecting group
GSRCSSDQVETGGSGGQNRICTCRPGW

SEQ ID NO: 78 - protein, 27 aa, synthetic construct
  SITE 2: note = Cys residue protected with ACM protecting group
  SITE 21: note = Cys residue protected with ACM protecting group
  SITE 27: note = Cys residue protected with ACM protecting group
SCGSRCSSDQVGGSGGRICTCRPGWYC

SEQ ID NO: 79 - protein, 27 aa, synthetic construct
  SITE 19: note = Cys residue protected with ACM protecting group
  SITE 25: note = Cys residue protected with ACM protecting group
GSRCSSDQVETGGSGGCTCRPGWYCAL

SEQ ID NO: 80 - protein, 27 aa, synthetic construct
  SITE 2: note = Cys residue protected with ACM protecting group
YCALSKQEGCRGGSGGRKCRPGFGVAR

SEQ ID NO: 81 - protein, 27 aa, synthetic construct
  SITE 8: note = Cys residue protected with ACM protecting group
KQEGCRLCAPLGGSGGPLRKCRPGFGV

SEQ ID NO: 82 - protein, 27 aa, synthetic construct
  SITE 11: note = Cys residue protected with ACM protecting group
ALSKQEGCRLCGGSGGRKCRPGFGVAR

SEQ ID NO: 83 - protein, 27 aa, synthetic construct
  SITE 2: note = Cys residue protected with ACM protecting group
  SITE 5: note = Cys residue protected with ACM protecting group
  SITE 20: note = Cys residue protected with ACM protecting group
  SITE 26: note = Cys residue protected with ACM protecting group
ECLSCGSRCSSGGSGGICTCRPGWYCA

SEQ ID NO: 84 - protein, 27 aa, synthetic construct
  SITE 11: note = Cys residue protected with ACM protecting group
  SITE 20: note = Cys residue protected with ACM protecting group
  SITE 26: note = Cys residue protected with ACM protecting group
CSSDQVETQACGGSGGICTCRPGWYCA

SEQ ID NO: 85 - protein, 27 aa, synthetic construct
  SITE 6: note = Cys residue protected with ACM protecting group
EGCRLCAPLRKGGSGGPLRKCRPGFGV

SEQ ID NO: 86 - protein, 27 aa, synthetic construct
  SITE 11: note = Cys residue protected with ACM protecting group
ALSKQEGCRLCGGSGGPLRKCRPGFGV

SEQ ID NO: 87 - protein, 27 aa, synthetic construct
  SITE 1: note = Cys residue protected with ACM protecting group
CALSKQEGCRLGGSGGRKCRPGFGVAR

SEQ ID NO: 88 - protein, 27 aa, synthetic construct
  SITE 1: note = Cys residue protected with ACM protecting group
  SITE 17: note = Cys residue protected with ACM protecting group
CALSKQEGCRLGGSGGCAPLRKCRPGF

SEQ ID NO: 89 - protein, 27 aa, synthetic construct
  SITE 1: note = Cys residue protected with ACM protecting group
  SITE 4: note = Cys residue protected with ACM protecting group
  SITE 21: note = Cys residue protected with ACM protecting group
  SITE 27: note = Cys residue protected with ACM protecting group
CLSCGSRCSSDGGSGGRICTCRPGWYC

SEQ ID NO: 90 - protein, 27 aa, synthetic construct
  SITE 10: note = Cys residue protected with ACM protecting group
LSKQEGCRLCAGGSGGPLRKCRPGFGV

SEQ ID NO: 91 - protein, 27 aa, synthetic construct
  SITE 9: note = Cys residue protected with ACM protecting group
SKQEGCRLCAPGGSGGRKCRPGFGVAR

SEQ ID NO: 92 - protein, 27 aa, synthetic construct
  SITE 8: note = Cys residue protected with ACM protecting group
KQEGCRLCAPLGGSGGRKCRPGFGVAR

SEQ ID NO: 93 - protein, 27 aa, synthetic construct
  SITE 7: note = Cys residue protected with ACM protecting group
QEGCRLCAPLRGGSGGRKCRPGFGVAR

SEQ ID NO: 94 - protein, 27 aa, synthetic construct
  SITE 1: note = Cys residue protected with ACM protecting group
CALSKQEGCRLGGSGGAPLRKCRPGFG

SEQ ID NO: 95 - protein, 27 aa, synthetic construct
  SITE 1: note = Cys residue protected with ACM protecting group
CALSKQEGCRLGGSGGPLRKCRPGFGV

SEQ ID NO: 96 - protein, 27 aa, synthetic construct
  SITE 20: note = Cys residue protected with ACM protecting group
  SITE 26: note = Cys residue protected with ACM protecting group
GSRCSSDQVETGGSGGICTCRPGWYCA

SEQ ID NO: 97 - protein, 27 aa, synthetic construct
  SITE 23: note = Cys residue protected with ACM protecting group
SRCSSDQVETQGGSGGQNRICTCRPGW

SEQ ID NO: 98 - protein, 27 aa, synthetic construct
  SITE 1: note = Cys residue protected with ACM protecting group
  SITE 20: note = Cys residue protected with ACM protecting group
  SITE 26: note = Cys residue protected with ACM protecting group
CGSRCSSDQVEGGSGGICTCRPGWYCA

SEQ ID NO: 99 - protein, 27 aa, synthetic construct
  SITE 2: note = Cys residue protected with ACM protecting group
  SITE 5: note = Cys residue protected with ACM protecting group
  SITE 22: note = Cys residue protected with ACM protecting group
ECLSCGSRCSSGGSGGNRICTCRPGWY

SEQ ID NO: 100 - protein, 27 aa, synthetic construct
  SITE 20: note = Cys residue protected with ACM protecting group
  SITE 26: note = Cys residue protected with ACM protecting group
SRCSSDQVETQGGSGGICTCRPGWYCA

SEQ ID NO: 101 - protein, 27 aa, synthetic construct
  SITE 2: note = Cys residue protected with ACM protecting group
YCALSKQEGCRGGSGGPLRKCRPGFGV

SEQ ID NO: 102 - protein, 27 aa, synthetic construct
  SITE 20: note = Cys residue protected with ACM protecting group
  SITE 26: note = Cys residue protected with ACM protecting group
RCSSDQVETQAGGSGGICTCRPGWYCA

SEQ ID NO: 103 - protein, 27 aa, synthetic construct
  SITE 9: note = Cys residue protected with ACM protecting group
SKQEGCRLCAPGGSGGPLRKCRPGFGV

SEQ ID NO: 104 - protein, 27 aa, synthetic construct
  SITE 2: note = Cys residue protected with ACM protecting group
  SITE 23: note = Cys residue protected with ACM protecting group
SCGSRCSSDQVGGSGGQNRICTCRPGW

SEQ ID NO: 105 - protein, 27 aa, synthetic construct
  SITE 6: note = Cys residue protected with ACM protecting group
EGCRLCAPLRKGGSGGRKCRPGFGVAR

SEQ ID NO: 106 - protein, 27 aa, synthetic construct
  SITE 1: note = Cys residue protected with ACM protecting group
  SITE 4: note = Cys residue protected with ACM protecting group
  SITE 23: note = Cys residue protected with ACM protecting group
CLSCGSRCSSDGGSGGQNRICTCRPGW

SEQ ID NO: 107 - protein, 27 aa, synthetic construct
  SITE 3: note = Cys residue protected with ACM protecting group
WYCALSKQEGCGGSGGPLRKCRPGFGV

SEQ ID NO: 108 - protein, 27 aa, synthetic construct
  SITE 7: note = Cys residue protected with ACM protecting group
QEGCRLCAPLRGGSGGAPLRKCRPGFG

SEQ ID NO: 109 - protein, 27 aa, synthetic construct
  SITE 3: note = Cys residue protected with ACM protecting group
  SITE 17: note = Cys residue protected with ACM protecting group
WYCALSKQEGCGGSGGCAPLRKCRPGF

SEQ ID NO: 110 - protein, 27 aa, synthetic construct
  SITE 11: note = Cys residue protected with ACM protecting group
ALSKQEGCRLCGGSGGAPLRKCRPGFG

SEQ ID NO: 111 - protein, 27 aa, synthetic construct
  SITE 6: note = Cys residue protected with ACM protecting group
EGCRLCAPLRKGGSGGAPLRKCRPGFG

SEQ ID NO: 112 - protein, 27 aa, synthetic construct
  SITE 2: note = Cys residue protected with ACM protecting group
  SITE 17: note = Cys residue protected with ACM protecting group
YCALSKQEGCRGGSGGCAPLRKCRPGF

SEQ ID NO: 113 - protein, 27 aa, synthetic construct
  SITE 3: note = Cys residue protected with ACM protecting group
  SITE 23: note = Cys residue protected with ACM protecting group
LSCGSRCSSDQGGSGGQNRICTCRPGW

SEQ ID NO: 114 - protein, 27 aa, synthetic construct
  SITE 10: note = Cys residue protected with ACM protecting group
LSKQEGCRLCAGGSGGAPLRKCRPGFG

SEQ ID NO: 115 - protein, 27 aa, synthetic construct
  SITE 22: note = Cys residue protected with ACM protecting group
RCSSDQVETQAGGSGGNRICTCRPGWY

SEQ ID NO: 116 - protein, 27 aa, synthetic construct
  SITE 8: note = Cys residue protected with ACM protecting group
KQEGCRLCAPLGGSGGAPLRKCRPGFG

SEQ ID NO: 117 - protein, 27 aa, synthetic construct
  SITE 9: note = Cys residue protected with ACM protecting group
SKQEGCRLCAPGGSGGAPLRKCRPGFG

SEQ ID NO: 118 - protein, 5 aa, Mus sp.
ADAAP

SEQ ID NO: 119 - protein, 5 aa, Homo sapiens
TVAAP

SEQ ID NO: 120 - protein, 11 aa, Mus sp.
ADAAPTVSIFP

SEQ ID NO: 121 - protein, 12 aa, Homo sapiens
TVAAPSVFIFPP

SEQ ID NO: 122 - protein, 6 aa, Homo sapiens
QPKAAP

SEQ ID NO: 123 - protein, 13 aa, Homo sapiens
QPKAAPSVTLFPP

SEQ ID NO: 124 - protein, 5 aa, synthetic construct
GGSGG

SEQ ID NO: 125 - protein, 9 aa, synthetic construct
GGSGGGGSG

SEQ ID NO: 126 - protein, 13 aa, synthetic construct
GGSGGGGSGGGGS

SEQ ID NO: 127 - protein, 6 aa, Mus sp.
AKTTAP

SEQ ID NO: 128 - protein, 6 aa, Homo sapiens
ASTKGP

SEQ ID NO: 129 - protein, 13 aa, Mus sp.
AKTTAPSVYPLAP

SEQ ID NO: 130 - protein, 13 aa, Homo sapiens
ASTKGPSVFPLAP

SEQ ID NO: 131 - protein, 6 aa, synthetic construct
GGGGSG

SEQ ID NO: 132 - protein, 10 aa, synthetic construct
GGGGSGGGGS

SEQ ID NO: 133 - protein, 14 aa, synthetic construct
GGGGSGGGGSGGGG

SEQ ID NO: 134 - protein, 27 aa, synthetic construct
  SITE 26: note = Cys residue protected with ACM protecting group
SRCSSDQVETQGGSGGTREQNRICTCR

SEQ ID NO: 135 - protein, 27 aa, synthetic construct
  SITE 26: note = Cys residue protected with ACM protecting group
RCSSDQVETQAGGSGGTREQNRICTCR

SEQ ID NO: 136 - protein, 27 aa, synthetic construct
  SITE 11: note = Cys residue protected with ACM protecting group
  SITE 26: note = Cys residue protected with ACM protecting group
CSSDQVETQACGGSGGTREQNRICTCR

SEQ ID NO: 137 - protein, 27 aa, synthetic construct
  SITE 4: note = Cys residue protected with ACM protecting group
  SITE 7: note = Cys residue protected with ACM protecting group
  SITE 25: note = Cys residue protected with ACM protecting group
VPECLSCGSRCGGSGGREQNRICTCRP

SEQ ID NO: 138 - protein, 27 aa, synthetic construct
  SITE 3: note = Cys residue protected with ACM protecting group
  SITE 6: note = Cys residue protected with ACM protecting group
  SITE 25: note = Cys residue protected with ACM protecting group
PECLSCGSRCSGGSGGREQNRICTCRP

SEQ ID NO: 139 - protein, 27 aa, synthetic construct
  SITE 2: note = Cys residue protected with ACM protecting group
  SITE 5: note = Cys residue protected with ACM protecting group
  SITE 25: note = Cys residue protected with ACM protecting group
ECLSCGSRCSSGGSGGREQNRICTCRP

SEQ ID NO: 140 - protein, 27 aa, synthetic construct
  SITE 1: note = Cys residue protected with ACM protecting group
  SITE 4: note = Cys residue protected with ACM protecting group
  SITE 25: note = Cys residue protected with ACM protecting group
CLSCGSRCSSDGGSGGREQNRICTCRP

SEQ ID NO: 141 - protein, 27 aa, synthetic construct
  SITE 3: note = Cys residue protected with ACM protecting group
  SITE 25: note = Cys residue protected with ACM protecting group
LSCGSRCSSDQGGSGGREQNRICTCRP

SEQ ID NO: 142 - protein, 27 aa, synthetic construct
  SITE 2: note = Cys residue protected with ACM protecting group
  SITE 25: note = Cys residue protected with ACM protecting group
SCGSRCSSDQVGGSGGREQNRICTCRP

SEQ ID NO: 143 - protein, 27 aa, synthetic construct
  SITE 1: note = Cys residue protected with ACM protecting group
  SITE 25: note = Cys residue protected with ACM protecting group
CGSRCSSDQVEGGSGGREQNRICTCRP

SEQ ID NO: 144 - protein, 27 aa, synthetic construct
  SITE 25: note = Cys residue protected with ACM protecting group
GSRCSSDQVETGGSGGREQNRICTCRP

SEQ ID NO: 145 - protein, 27 aa, synthetic construct
  SITE 25: note = Cys residue protected with ACM protecting group
SRCSSDQVETQGGSGGREQNRICTCRP

SEQ ID NO: 146 - protein, 27 aa, synthetic construct
  SITE 25: note = Cys residue protected with ACM protecting group
RCSSDQVETQAGGSGGREQNRICTCRP

SEQ ID NO: 147 - protein, 27 aa, synthetic construct
  SITE 11: note = Cys residue protected with ACM protecting group
  SITE 25: note = Cys residue protected with ACM protecting group
CSSDQVETQACGGSGGREQNRICTCRP

SEQ ID NO: 148 - protein, 27 aa, synthetic construct
  SITE 4: note = Cys residue protected with ACM protecting group
  SITE 7: note = Cys residue protected with ACM protecting group
  SITE 24: note = Cys residue protected with ACM protecting group
VPECLSCGSRCGGSGGEQNRICTCRPG

SEQ ID NO: 149 - protein, 27 aa, synthetic construct
  SITE 3: note = Cys residue protected with ACM protecting group
  SITE 6: note = Cys residue protected with ACM protecting group
  SITE 24: note = Cys residue protected with ACM protecting group
PECLSCGSRCSGGSGGEQNRICTCRPG

SEQ ID NO: 150 - protein, 27 aa, synthetic construct
  SITE 2: note = Cys residue protected with ACM protecting group
  SITE 5: note = Cys residue protected with ACM protecting group
  SITE 24: note = Cys residue protected with ACM protecting group
ECLSCGSRCSSGGSGGEQNRICTCRPG

SEQ ID NO: 151 - protein, 27 aa, synthetic construct
  SITE 1: note = Cys residue protected with ACM protecting group
  SITE 4: note = Cys residue protected with ACM protecting group
  SITE 24: note = Cys residue protected with ACM protecting group
CLSCGSRCSSDGGSGGEQNRICTCRPG

SEQ ID NO: 152 - protein, 27 aa, synthetic construct
  SITE 3: note = Cys residue protected with ACM protecting group
  SITE 24: note = Cys residue protected with ACM protecting group
LSCGSRCSSDQGGSGGEQNRICTCRPG

SEQ ID NO: 153 - protein, 27 aa, synthetic construct
  SITE 2: note = Cys residue protected with ACM protecting group
  SITE 24: note = Cys residue protected with ACM protecting group
SCGSRCSSDQVGGSGGEQNRICTCRPG

SEQ ID NO: 154 - protein, 27 aa, synthetic construct
  SITE 1: note = Cys residue protected with ACM protecting group
  SITE 24: note = Cys residue protected with ACM protecting group
CGSRCSSDQVEGGSGGEQNRICTCRPG

SEQ ID NO: 155 - protein, 27 aa, synthetic construct
  SITE 24: note = Cys residue protected with ACM protecting group
GSRCSSDQVETGGSGGEQNRICTCRPG

SEQ ID NO: 156 - protein, 27 aa, synthetic construct
  SITE 24: note = Cys residue protected with ACM protecting group
SRCSSDQVETQGGSGGEQNRICTCRPG

SEQ ID NO: 157 - protein, 27 aa, synthetic construct
  SITE 24: note = Cys residue protected with ACM protecting group
RCSSDQVETQAGGSGGEQNRICTCRPG

SEQ ID NO: 158 - protein, 27 aa, synthetic construct
  SITE 11: note = Cys residue protected with ACM protecting group
  SITE 24: note = Cys residue protected with ACM protecting group
CSSDQVETQACGGSGGEQNRICTCRPG

SEQ ID NO: 159 - protein, 27 aa, synthetic construct
  SITE 4: note = Cys residue protected with ACM protecting group
  SITE 7: note = Cys residue protected with ACM protecting group
  SITE 23: note = Cys residue protected with ACM protecting group
VPECLSCGSRCGGSGGQNRICTCRPGW

SEQ ID NO: 160 - protein, 27 aa, synthetic construct
  SITE 3: note = Cys residue protected with ACM protecting group
  SITE 6: note = Cys residue protected with ACM protecting group
  SITE 23: note = Cys residue protected with ACM protecting group
PECLSCGSRCSGGSGGQNRICTCRPGW

SEQ ID NO: 161 - protein, 27 aa, synthetic construct
  SITE 2: note = Cys residue protected with ACM protecting group
  SITE 5: note = Cys residue protected with ACM protecting group
  SITE 23: note = Cys residue protected with ACM protecting group
ECLSCGSRCSSGGSGGQNRICTCRPGW

SEQ ID NO: 162 - protein, 27 aa, synthetic construct
  SITE 1: note = Cys residue protected with ACM protecting group
  SITE 4: note = Cys residue protected with ACM protecting group
  SITE 23: note = Cys residue protected with ACM protecting group
CLSCGSRCSSDGGSGGQNRICTCRPGW

SEQ ID NO: 163 - protein, 27 aa, synthetic construct
  SITE 3: note = Cys residue protected with ACM protecting group
  SITE 23: note = Cys residue protected with ACM protecting group
LSCGSRCSSDQGGSGGQNRICTCRPGW

SEQ ID NO: 164 - protein, 27 aa, synthetic construct
  SITE 2: note = Cys residue protected with ACM protecting group
  SITE 23: note = Cys residue protected with ACM protecting group
SCGSRCSSDQVGGSGGQNRICTCRPGW

SEQ ID NO: 165 - protein, 27 aa, synthetic construct
  SITE 1: note = Cys residue protected with ACM protecting group
  SITE 23: note = Cys residue protected with ACM protecting group
CGSRCSSDQVEGGSGGQNRICTCRPGW

SEQ ID NO: 166 - protein, 27 aa, synthetic construct
  SITE 23: note = Cys residue protected with ACM protecting group
GSRCSSDQVETGGSGGQNRICTCRPGW

SEQ ID NO: 167 - protein, 27 aa, synthetic construct
  SITE 23: note = Cys residue protected with ACM protecting group
SRCSSDQVETQGGSGGQNRICTCRPGW

SEQ ID NO: 168 - protein, 27 aa, synthetic construct
  SITE 23: note = Cys residue protected with ACM protecting group
RCSSDQVETQAGGSGGQNRICTCRPGW

SEQ ID NO: 169 - protein, 27 aa, synthetic construct
  SITE 11: note = Cys residue protected with ACM protecting group
  SITE 23: note = Cys residue protected with ACM protecting group
CSSDQVETQACGGSGGQNRICTCRPGW

SEQ ID NO: 170 - protein, 27 aa, synthetic construct
  SITE 4: note = Cys residue protected with ACM protecting group
  SITE 7: note = Cys residue protected with ACM protecting group
  SITE 22: note = Cys residue protected with ACM protecting group
VPECLSCGSRCGGSGGNRICTCRPGWY

SEQ ID NO: 171 - protein, 27 aa, synthetic construct
  SITE 3: note = Cys residue protected with ACM protecting group
  SITE 6: note = Cys residue protected with ACM protecting group
  SITE 22: note = Cys residue protected with ACM protecting group
PECLSCGSRCSGGSGGNRICTCRPGWY

SEQ ID NO: 172 - protein, 27 aa, synthetic construct
  SITE 2: note = Cys residue protected with ACM protecting group
  SITE 5: note = Cys residue protected with ACM protecting group
  SITE 22: note = Cys residue protected with ACM protecting group
ECLSCGSRCSSGGSGGNRICTCRPGWY

SEQ ID NO: 173 - protein, 27 aa, synthetic construct
  SITE 1: note = Cys residue protected with ACM protecting group
  SITE 4: note = Cys residue protected with ACM protecting group
  SITE 22: note = Cys residue protected with ACM protecting group
CLSCGSRCSSDGGSGGNRICTCRPGWY

SEQ ID NO: 174 - protein, 27 aa, synthetic construct
  SITE 3: note = Cys residue protected with ACM protecting group
  SITE 22: note = Cys residue protected with ACM protecting group
LSCGSRCSSDQGGSGGNRICTCRPGWY

SEQ ID NO: 175 - protein, 27 aa, synthetic construct
  SITE 2: note = Cys residue protected with ACM protecting group
  SITE 22: note = Cys residue protected with ACM protecting group
SCGSRCSSDQVGGSGGNRICTCRPGWY

SEQ ID NO: 176 - protein, 27 aa, synthetic construct
  SITE 1: note = Cys residue protected with ACM protecting group
  SITE 22: note = Cys residue protected with ACM protecting group
CGSRCSSDQVEGGSGGNRICTCRPGWY

SEQ ID NO: 177 - protein, 27 aa, synthetic construct
  SITE 22: note = Cys residue protected with ACM protecting group
GSRCSSDQVETGGSGGNRICTCRPGWY

SEQ ID NO: 178 - protein, 27 aa, synthetic construct
  SITE 22: note = Cys residue protected with ACM protecting group
SRCSSDQVETQGGSGGNRICTCRPGWY

SEQ ID NO: 179 - protein, 27 aa, synthetic construct
  SITE 22: note = Cys residue protected with ACM protecting group
RCSSDQVETQAGGSGGNRICTCRPGWY

SEQ ID NO: 180 - protein, 27 aa, synthetic construct
  SITE 11: note = Cys residue protected with ACM protecting group
  SITE 22: note = Cys residue protected with ACM protecting group
CSSDQVETQACGGSGGNRICTCRPGWY

SEQ ID NO: 181 - protein, 27 aa, synthetic construct
  SITE 4: note = Cys residue protected with ACM protecting group
  SITE 7: note = Cys residue protected with ACM protecting group
  SITE 21: note = Cys residue protected with ACM protecting group
  SITE 27: note = Cys residue protected with ACM protecting group
VPECLSCGSRCGGSGGRICTCRPGWYC

SEQ ID NO: 182 - protein, 27 aa, synthetic construct
  SITE 3: note = Cys residue protected with ACM protecting group
  SITE 6: note = Cys residue protected with ACM protecting group
  SITE 21: note = Cys residue protected with ACM protecting group
  SITE 27: note = Cys residue protected with ACM protecting group
PECLSCGSRCSGGSGGRICTCRPGWYC

SEQ ID NO: 183 - protein, 27 aa, synthetic construct
  SITE 2: note = Cys residue protected with ACM protecting group
  SITE 5: note = Cys residue protected with ACM protecting group
  SITE 21: note = Cys residue protected with ACM protecting group
  SITE 27: note = Cys residue protected with ACM protecting group
ECLSCGSRCSSGGSGGRICTCRPGWYC

SEQ ID NO: 184 - protein, 27 aa, synthetic construct
  SITE 1: note = Cys residue protected with ACM protecting group
  SITE 4: note = Cys residue protected with ACM protecting group
  SITE 21: note = Cys residue protected with ACM protecting group
  SITE 27: note = Cys residue protected with ACM protecting group
CLSCGSRCSSDGGSGGRICTCRPGWYC

SEQ ID NO: 185 - protein, 27 aa, synthetic construct
  SITE 3: note = Cys residue protected with ACM protecting group
  SITE 21: note = Cys residue protected with ACM protecting group
  SITE 27: note = Cys residue protected with ACM protecting group
LSCGSRCSSDQGGSGGRICTCRPGWYC

SEQ ID NO: 186 - protein, 27 aa, synthetic construct
  SITE 2: note = Cys residue protected with ACM protecting group
  SITE 21: note = Cys residue protected with ACM protecting group
  SITE 27: note = Cys residue protected with ACM protecting group
SCGSRCSSDQVGGSGGRICTCRPGWYC

SEQ ID NO: 187 - protein, 27 aa, synthetic construct
  SITE 1: note = Cys residue protected with ACM protecting group
  SITE 21: note = Cys residue protected with ACM protecting group
  SITE 27: note = Cys residue protected with ACM protecting group
CGSRCSSDQVEGGSGGRICTCRPGWYC

SEQ ID NO: 188 - protein, 27 aa, synthetic construct
  SITE 21: note = Cys residue protected with ACM protecting group
  SITE 27: note = Cys residue protected with ACM protecting group
GSRCSSDQVETGGSGGRICTCRPGWYC

SEQ ID NO: 189 - protein, 27 aa, synthetic construct
  SITE 21: note = Cys residue protected with ACM protecting group
  SITE 27: note = Cys residue protected with ACM protecting group
SRCSSDQVETQGGSGGRICTCRPGWYC

SEQ ID NO: 190 - protein, 27 aa, synthetic construct
  SITE 21: note = Cys residue protected with ACM protecting group
  SITE 27: note = Cys residue protected with ACM protecting group
RCSSDQVETQAGGSGGRICTCRPGWYC

SEQ ID NO: 191 - protein, 27 aa, synthetic construct
  SITE 11: note = Cys residue protected with ACM protecting group
  SITE 21: note = Cys residue protected with ACM protecting group
  SITE 27: note = Cys residue protected with ACM protecting group
CSSDQVETQACGGSGGRICTCRPGWYC

SEQ ID NO: 192 - protein, 27 aa, synthetic construct
  SITE 4: note = Cys residue protected with ACM protecting group
  SITE 7: note = Cys residue protected with ACM protecting group
  SITE 20: note = Cys residue protected with ACM protecting group
  SITE 26: note = Cys residue protected with ACM protecting group
VPECLSCGSRCGGSGGICTCRPGWYCA

SEQ ID NO: 193 - protein, 27 aa, synthetic construct
  SITE 3: note = Cys residue protected with ACM protecting group
  SITE 6: note = Cys residue protected with ACM protecting group
  SITE 20: note = Cys residue protected with ACM protecting group
  SITE 26: note = Cys residue protected with ACM protecting group
PECLSCGSRCSGGSGGICTCRPGWYCA

SEQ ID NO: 194 - protein, 27 aa, synthetic construct
  SITE 2: note = Cys residue protected with ACM protecting group
  SITE 5: note = Cys residue protected with ACM protecting group
  SITE 20: note = Cys residue protected with ACM protecting group
  SITE 26: note = Cys residue protected with ACM protecting group
ECLSCGSRCSSGGSGGICTCRPGWYCA

SEQ ID NO: 195 - protein, 27 aa, synthetic construct
  SITE 1: note = Cys residue protected with ACM protecting group
  SITE 20: note = Cys residue protected with ACM protecting group
  SITE 26: note = Cys residue protected with ACM protecting group
CGSRCSSDQVEGGSGGICTCRPGWYCA

SEQ ID NO: 196 - protein, 27 aa, synthetic construct
  SITE 20: note = Cys residue protected with ACM protecting group
  SITE 26: note = Cys residue protected with ACM protecting group
GSRCSSDQVETGGSGGICTCRPGWYCA

SEQ ID NO: 197 - protein, 27 aa, synthetic construct
  SITE 20: note = Cys residue protected with ACM protecting group
  SITE 26: note = Cys residue protected with ACM protecting group
SRCSSDQVETQGGSGGICTCRPGWYCA

SEQ ID NO: 198 - protein, 27 aa, synthetic construct
  SITE 20: note = Cys residue protected with ACM protecting group
  SITE 26: note = Cys residue protected with ACM protecting group
RCSSDQVETQAGGSGGICTCRPGWYCA

SEQ ID NO: 199 - protein, 27 aa, synthetic construct
  SITE 11: note = Cys residue protected with ACM protecting group
  SITE 20: note = Cys residue protected with ACM protecting group
  SITE 26: note = Cys residue protected with ACM protecting group
CSSDQVETQACGGSGGICTCRPGWYCA

SEQ ID NO: 200 - protein, 27 aa, synthetic construct
  SITE 4: note = Cys residue protected with ACM protecting group
  SITE 7: note = Cys residue protected with ACM protecting group
  SITE 19: note = Cys residue protected with ACM protecting group
  SITE 25: note = Cys residue protected with ACM protecting group
VPECLSCGSRCGGSGGCTCRPGWYCAL

SEQ ID NO: 201 - protein, 27 aa, synthetic construct
  SITE 3: note = Cys residue protected with ACM protecting group
  SITE 6: note = Cys residue protected with ACM protecting group
  SITE 19: note = Cys residue protected with ACM protecting group
  SITE 25: note = Cys residue protected with ACM protecting group
PECLSCGSRCSGGSGGCTCRPGWYCAL

SEQ ID NO: 202 - protein, 27 aa, synthetic construct
  SITE 2: note = Cys residue protected with ACM protecting group
  SITE 5: note = Cys residue protected with ACM protecting group
  SITE 19: note = Cys residue protected with ACM protecting group
  SITE 25: note = Cys residue protected with ACM protecting group
ECLSCGSRCSSGGSGGCTCRPGWYCAL

SEQ ID NO: 203 - protein, 27 aa, synthetic construct
  SITE 1: note = Cys residue protected with ACM protecting group
  SITE 4: note = Cys residue protected with ACM protecting group
  SITE 19: note = Cys residue protected with ACM protecting group
  SITE 25: note = Cys residue protected with ACM protecting group
CLSCGSRCSSDGGSGGCTCRPGWYCAL

SEQ ID NO: 204 - protein, 27 aa, synthetic construct
  SITE 3: note = Cys residue protected with ACM protecting group
  SITE 19: note = Cys residue protected with ACM protecting group
  SITE 25: note = Cys residue protected with ACM protecting group
LSCGSRCSSDQGGSGGCTCRPGWYCAL

SEQ ID NO: 205 - protein, 27 aa, synthetic construct
  SITE 2: note = Cys residue protected with ACM protecting group
  SITE 19: note = Cys residue protected with ACM protecting group
  SITE 25: note = Cys residue protected with ACM protecting group
SCGSRCSSDQVGGSGGCTCRPGWYCAL

SEQ ID NO: 206 - protein, 27 aa, synthetic construct
  SITE 1: note = Cys residue protected with ACM protecting group
  SITE 19: note = Cys residue protected with ACM protecting group
  SITE 25: note = Cys residue protected with ACM protecting group
CGSRCSSDQVEGGSGGCTCRPGWYCAL

SEQ ID NO: 207 - protein, 27 aa, synthetic construct
  SITE 19: note = Cys residue protected with ACM protecting group
  SITE 25: note = Cys residue protected with ACM protecting group
GSRCSSDQVETGGSGGCTCRPGWYCAL

SEQ ID NO: 208 - protein, 27 aa, synthetic construct
  SITE 19: note = Cys residue protected with ACM protecting group
  SITE 25: note = Cys residue protected with ACM protecting group
SRCSSDQVETQGGSGGCTCRPGWYCAL

SEQ ID NO: 209 - protein, 27 aa, synthetic construct
  SITE 19: note = Cys residue protected with ACM protecting group
  SITE 25: note = Cys residue protected with ACM protecting group
RCSSDQVETQAGGSGGCTCRPGWYCAL

SEQ ID NO: 210 - protein, 27 aa, synthetic construct
  SITE 11: note = Cys residue protected with ACM protecting group
  SITE 19: note = Cys residue protected with ACM protecting group
  SITE 25: note = Cys residue protected with ACM protecting group
CSSDQVETQACGGSGGCTCRPGWYCAL

SEQ ID NO: 211 - protein, 27 aa, synthetic construct
  SITE 1: note = Cys residue protected with ACM protecting group
  SITE 9: note = Cys residue protected with ACM protecting group
CTREQNRICTCGGSGGRPGWYCALSKQ

SEQ ID NO: 212 - protein, 27 aa, synthetic construct
  SITE 8: note = Cys residue protected with ACM protecting group
TREQNRICTCRGGSGGRPGWYCALSKQ

SEQ ID NO: 213 - protein, 27 aa, synthetic construct
  SITE 7: note = Cys residue protected with ACM protecting group
REQNRICTCRPGGSGGRPGWYCALSKQ

SEQ ID NO: 214 - protein, 27 aa, synthetic construct
  SITE 6: note = Cys residue protected with ACM protecting group
EQNRICTCRPGGGSGGRPGWYCALSKQ

SEQ ID NO: 215 - protein, 27 aa, synthetic construct
  SITE 5: note = Cys residue protected with ACM protecting group
QNRICTCRPGWGGSGGRPGWYCALSKQ

SEQ ID NO: 216 - protein, 27 aa, synthetic construct
  SITE 4: note = Cys residue protected with ACM protecting group
NRICTCRPGWYGGSGGRPGWYCALSKQ

SEQ ID NO: 217 - protein, 27 aa, synthetic construct
  SITE 3: note = Cys residue protected with ACM protecting group
  SITE 17: note = Cys residue protected with ACM protecting group
WYCALSKQEGCGGSGGCAPLRKCRPGF

SEQ ID NO: 218 - protein, 27 aa, synthetic construct
  SITE 2: note = Cys residue protected with ACM protecting group
  SITE 17: note = Cys residue protected with ACM protecting group
YCALSKQEGCRGGSGGCAPLRKCRPGF

SEQ ID NO: 219 - protein, 27 aa, synthetic construct
  SITE 1: note = Cys residue protected with ACM protecting group
  SITE 17: note = Cys residue protected with ACM protecting group
CALSKQEGCRLGGSGGCAPLRKCRPGF

SEQ ID NO: 220 - protein, 27 aa, synthetic construct
  SITE 11: note = Cys residue protected with ACM protecting group
  SITE 17: note = Cys residue protected with ACM protecting group
ALSKQEGCRLCGGSGGCAPLRKCRPGF

SEQ ID NO: 221 - protein, 27 aa, synthetic construct
  SITE 10: note = Cys residue protected with ACM protecting group
  SITE 17: note = Cys residue protected with ACM protecting group
LSKQEGCRLCAGGSGGCAPLRKCRPGF

SEQ ID NO: 222 - protein, 27 aa, synthetic construct
  SITE 9: note = Cys residue protected with ACM protecting group
  SITE 17: note = Cys residue protected with ACM protecting group
SKQEGCRLCAPGGSGGCAPLRKCRPGF

SEQ ID NO: 223 - protein, 27 aa, synthetic construct
  SITE 8: note = Cys residue protected with ACM protecting group
  SITE 17: note = Cys residue protected with ACM protecting group
KQEGCRLCAPLGGSGGCAPLRKCRPGF

SEQ ID NO: 224 - protein, 27 aa, synthetic construct
  SITE 7: note = Cys residue protected with ACM protecting group
  SITE 17: note = Cys residue protected with ACM protecting group
QEGCRLCAPLRGGSGGCAPLRKCRPGF

SEQ ID NO: 225 - protein, 27 aa, synthetic construct
  SITE 6: note = Cys residue protected with ACM protecting group
  SITE 17: note = Cys residue protected with ACM protecting group
EGCRLCAPLRKGGSGGCAPLRKCRPGF

SEQ ID NO: 226 - protein, 27 aa, synthetic construct
  SITE 3: note = Cys residue protected with ACM protecting group
WYCALSKQEGCGGSGGAPLRKCRPGFG

SEQ ID NO: 227 - protein, 27 aa, synthetic construct
  SITE 2: note = Cys residue protected with ACM protecting group
YCALSKQEGCRGGSGGAPLRKCRPGFG

SEQ ID NO: 228 - protein, 27 aa, synthetic construct
  SITE 1: note = Cys residue protected with ACM protecting group
CALSKQEGCRLGGSGGAPLRKCRPGFG

SEQ ID NO: 229 - protein, 27 aa, synthetic construct
  SITE 11: note = Cys residue protected with ACM protecting group
ALSKQEGCRLCGGSGGAPLRKCRPGFG

SEQ ID NO: 230 - protein, 27 aa, synthetic construct
  SITE 10: note = Cys residue protected with ACM protecting group
LSKQEGCRLCAGGSGGAPLRKCRPGFG

SEQ ID NO: 231 - protein, 27 aa, synthetic construct
  SITE 9: note = Cys residue protected with ACM protecting group
SKQEGCRLCAPGGSGGAPLRKCRPGFG

SEQ ID NO: 232 - protein, 27 aa, synthetic construct
  SITE 8: note = Cys residue protected with ACM protecting group
KQEGCRLCAPLGGSGGAPLRKCRPGFG

SEQ ID NO: 233 - protein, 27 aa, synthetic construct
  SITE 7: note = Cys residue protected with ACM protecting group
QEGCRLCAPLRGGSGGAPLRKCRPGFG

SEQ ID NO: 234 - protein, 27 aa, synthetic construct
  SITE 6: note = Cys residue protected with ACM protecting group
EGCRLCAPLRKGGSGGAPLRKCRPGFG

SEQ ID NO: 235 - protein, 27 aa, synthetic construct
  SITE 3: note = Cys residue protected with ACM protecting group
WYCALSKQEGCGGSGGPLRKCRPGFGV

SEQ ID NO: 236 - protein, 27 aa, synthetic construct
  SITE 2: note = Cys residue protected with ACM protecting group
YCALSKQEGCRGGSGGPLRKCRPGFGV

SEQ ID NO: 237 - protein, 27 aa, synthetic construct
  SITE 1: note = Cys residue protected with ACM protecting group
CALSKQEGCRLGGSGGPLRKCRPGFGV

SEQ ID NO: 238 - protein, 27 aa, synthetic construct
  SITE 11: note = Cys residue protected with ACM protecting group
ALSKQEGCRLCGGSGGPLRKCRPGFGV

SEQ ID NO: 239 - protein, 27 aa, synthetic construct
  SITE 10: note = Cys residue protected with ACM protecting group
LSKQEGCRLCAGGSGGPLRKCRPGFGV

SEQ ID NO: 240 - protein, 27 aa, synthetic construct
  SITE 9: note = Cys residue protected with ACM protecting group
SKQEGCRLCAPGGSGGPLRKCRPGFGV

SEQ ID NO: 241 - protein, 27 aa, synthetic construct
  SITE 8: note = Cys residue protected with ACM protecting group
KQEGCRLCAPLGGSGGPLRKCRPGFGV

SEQ ID NO: 242 - protein, 27 aa, synthetic construct
  SITE 7: note = Cys residue protected with ACM protecting group
QEGCRLCAPLRGGSGGPLRKCRPGFGV

SEQ ID NO: 243 - protein, 27 aa, synthetic construct
  SITE 6: note = Cys residue protected with ACM protecting group
EGCRLCAPLRKGGSGGPLRKCRPGFGV

SEQ ID NO: 244 - protein, 27 aa, synthetic construct
  SITE 3: note = Cys residue protected with ACM protecting group
WYCALSKQEGCGGSGGLRKCRPGFGVA

SEQ ID NO: 245 - protein, 27 aa, synthetic construct
  SITE 2: note = Cys residue protected with ACM protecting group
YCALSKQEGCRGGSGGRKCRPGFGVAR

SEQ ID NO: 246 - protein, 27 aa, synthetic construct
  SITE 1: note = Cys residue protected with ACM protecting group
CALSKQEGCRLGGSGGRKCRPGFGVAR

SEQ ID NO: 247 - protein, 27 aa, synthetic construct
  SITE 11: note = Cys residue protected with ACM protecting group
ALSKQEGCRLCGGSGGRKCRPGFGVAR

SEQ ID NO: 248 - protein, 27 aa, synthetic construct
  SITE 10: note = Cys residue protected with ACM protecting group
LSKQEGCRLCAGGSGGRKCRPGFGVAR

SEQ ID NO: 249 - protein, 27 aa, synthetic construct
  SITE 9: note = Cys residue protected with ACM protecting group
SKQEGCRLCAPGGSGGRKCRPGFGVAR

SEQ ID NO: 250 - protein, 27 aa, synthetic construct
  SITE 8: note = Cys residue protected with ACM protecting group
KQEGCRLCAPLGGSGGRKCRPGFGVAR

SEQ ID NO: 251 - protein, 27 aa, synthetic construct
  SITE 7: note = Cys residue protected with ACM protecting group
QEGCRLCAPLRGGSGGRKCRPGFGVAR

SEQ ID NO: 252 - protein, 27 aa, synthetic construct
  SITE 6: note = Cys residue protected with ACM protecting group
EGCRLCAPLRKGGSGGRKCRPGFGVAR

SEQ ID NO: 253 - protein, 20 aa, Homo sapiens
REQNRICTCRPGWYCALSKQ

SEQ ID NO: 254 - protein, 20 aa, Homo sapiens
CRPGWYCALSKQEGCRLCAP

SEQ ID NO: 255 - protein, 20 aa, Homo sapiens
LSKQEGCRLCAPLRKCRPGF

SEQ ID NO: 256 - protein, 20 aa, Homo sapiens
LCAPLRKCRPGFGVARPGTE

SEQ ID NO: 257 - protein, 8 aa, Mus sp.
GYTFTDYJ

SEQ ID NO: 258 - protein, 8 aa, Mus sp.
VDPEYGST

SEQ ID NO: 259 - protein, 14 aa, Mus sp.
ARDDGSYSPFDYWG

SEQ ID NO: 260 - protein, 6 aa, Mus sp.
QNINKY

SEQ ID NO: 261 - protein, 9 aa, Mus sp.
CLQYVNLJT

SEQ ID NO: 262 - protein, 4 aa, Mus sp.
LLIR

SEQ ID NO: 263 - protein, 6 aa, synthetic construct
  VARIANT 4: note = Gly or Ala
  VARIANT 5: note = Asn, Gln, Ser or Thr
SSGXXY

SEQ ID NO: 264 - protein, 8 aa, synthetic construct
  VARIANT 6: note = Gly or Ala
  VARIANT 7: note = Asn, Gln, Ser or Thr
VDPEYXXT

SEQ ID NO: 265 - protein, 14 aa, synthetic construct
  VARIANT 2: note = Arg, Lys or His
  VARIANT 4: note = Asp or Glu
  VARIANT 5: note = Gly or Ala
  VARIANT 7: note = Asn, Gln, Ser or Thr
  VARIANT 9: note = Ala, Val, Leu, Ile, Pro, Met, Trp, Phe or Tyr
  VARIANT 12: note = Ala, Val, Leu, Ile, Pro, Met, Trp, Phe or Tyr
  VARIANT 13: note = Asp or Glu
  VARIANT 14: note = Ala, Val, Leu, Ile, Pro, Met, Trp, Phe or Tyr
QXVXXYXSXWYXXX

SEQ ID NO: 266 - protein, 14 aa, synthetic construct
  VARIANT 2: note = Lys, Arg or His
  VARIANT 4: note = Asp or Glu
  VARIANT 5: note = Gly or Ala
  VARIANT 6: note = Asn, Gln, Ser or Thr
  VARIANT 7: note = Ala, Val, Leu, Ile, Pro, Met, Trp, Phe or Tyr
  VARIANT 10: note = Ala, Val, Leu, Ile, Pro, Met, Trp, Phe or Tyr
  VARIANT 11: note = Asp or Glu
  VARIANT 12: note = Ala, Val, Leu, Ile, Pro, Met, Trp, Phe or Tyr
AXDXXXXSPXXXWG

SEQ ID NO: 267 - protein, 10 aa, synthetic construct
  VARIANT 10: note = Ala, Val, Leu, Ile, Pro, Met, Trp, Phe or Tyr
SASSSVYYMX

SEQ ID NO: 268 - protein, 6 aa, synthetic construct
  VARIANT 6: note = Ala, Val, Leu, Ile, Pro, Met, Trp, Phe or Tyr
QNINKX

SEQ ID NO: 269 - protein, 7 aa, synthetic construct
  VARIANT 7: note = Asn, Gln, Ser or Thr
STSNLAX

SEQ ID NO: 270 - protein, 9 aa, synthetic construct
  VARIANT 6: note = Ala, Val, Leu, Ile, Pro, Met, Trp, Phe or Tyr
  VARIANT 9: note = Asn, Gln, Ser or Thr
QQRRNXPYX

SEQ ID NO: 271 - protein, 9 aa, synthetic construct
  VARIANT 4: note = Ala, Val, Leu, Ile, Pro, Met, Trp, Phe or Tyr
  VARIANT 8: note = Leu or Ile
  VARIANT 9: note = Asn, Gln, Ser or Thr
CLQXVNLXX

SEQ ID NO: 272 - protein, 9 aa, Mus sp.
CLQYVNLLT

SEQ ID NO: 273 - protein, 9 aa, Mus sp.
CLQYVNLIT

SEQ ID NO: 274 - protein, 8 aa, Mus sp.
GYTFTDYL

SEQ ID NO: 275 - protein, 8 aa, Mus sp.
GYTFTDYI

SEQ ID NO: 276 - protein, 7 aa, synthetic construct
  VARIANT 2: note = any amino acid
  VARIANT 5: note = any amino acid
  VARIANT 6: note = any amino acid
GXTFXXY

SEQ ID NO: 277 - protein, 8 aa, synthetic construct
  VARIANT 2: note = any amino acid
  VARIANT 5: note = any amino acid
  VARIANT 6: note = any amino acid
  VARIANT 8: note = any amino acid
GXTFXXYX

SEQ ID NO: 278 - protein, 14 aa, synthetic construct
  VARIANT 1: note = any amino acid
  VARIANT 3: note = any amino acid
  VARIANT 6: note = any amino acid
  VARIANT 8: note = any amino acid
  VARIANT 10: note = any amino acid
  VARIANT 11: note = any amino acid
  VARIANT 14: note = any amino acid
XRXDGXSXYXXFDX

SEQ ID NO: 279 - protein, 14 aa, synthetic construct
  VARIANT 1: note = any amino acid
  VARIANT 3: note = any amino acid
  VARIANT 8: note = any amino acid
  VARIANT 9: note = any amino acid
  VARIANT 12: note = any amino acid
  VARIANT 13: note = any amino acid
  VARIANT 14: note = any amino acid
XRXDGSYXXFDXXX

SEQ ID NO: 280 - protein, 459 aa, Bos taurus
MAPTAFWAALAVGLQFWAAGRAVPAQAVFTPYIPEPGSSCRQQEYYNQKIQMCCSKCPPGYRVQSLCNMTLDTICASCESSTYTQLWNLVTACFSCNSRCSSDQVETQACTTKQNRICTCKPGWYCTLGRQEGCRLCVALRKCGPGFGVAKPGTATTNVICAPCGPGTFSDTTSYTDTCKPHRNCSSVAIPGTASTDAVCTSVLPTRKVARGPATTRSQHMEPTLGPSTAPSTFFLLPKVPSPPSSPVEQPNTGNISLPIELIVGVTALGLLLIVVVNCVIMTQKKKKPFCLQGDAKVPHLPANKAQGAPGPEQQHLLTTAPSSSSSSLESSTSSTDKRAPTRSQLQSPGVEKASTSGEAQTGCSSSEASSGGHGTQVNVTCIVNVCSGPDHSSQCPSQAGSTRDTDASTPNSPKEEQVPFSKEERPFQSQPGAPETLLQGLEEKPLPLGVPDAGMKPS

SEQ ID NO: 281 - protein, 458 aa, Bison bison
MAPTAFWAALAVGLQFWAAGRAVPAQAVFTPYIPEPGSSCRQQEYYNHKIQMCCSKCPPGYRVQSLCNTTLDTICASCESSTYTQLWNLVTACFSCNSRCSSDQVETQACTTKQNRICTCKPGWYCTLGRQEGCRLCVALRKCGPGFGVAKPGTATTNVICAPCGPGTFSDTTSYTDTCKPHRNCSSVAIPGTASTDAVCTSVLPTRKVARGPATTRSQHMEPTLGPSTAPSTFFLLPKVPSPPSSPVEQPNAGNISLPIELIVGVTALGLLLIVVVNCVIMTQKKKKPFCLQGDAKVPHLPANKAQGAPGPEQQHLLTTAPSSSSSSLESSTSSTDKRAPTRSQLQSPGVEANTSGEAQTGCSSSEASSGGHGTQVNVTCIVNVCSGPDHSSQCPSQAGSTRDTDASTPNSPKEEQVPFSKEERPFQSQPGAPETLLQGLEEKPLPLGVPDAGMKPS

SEQ ID NO: 282 - protein, 474 aa, Mus musculus
MAPAALWVALVFELQLWATGHTVPAQVVLTPYKPEPGYECQISQEYYDRKAQMCCAKCPPGQYVKHFCNKTSDTVCADCEASMYTQVWNQFRTCLSCSSSCTTDQVEIRACTKQQNRVCACEAGRYCALKTHSGSCRQCMRLSKCGPGFGVASSRAPNGNVLCKACAPGTFSDTTSSTDVCRPHRICSILAIPGNASTDAVCAPESPTLSAIPRTLYVSQPEPTRSQPLDQEPGPSQTPSILTSLGSTPIIEQSTKGGISLPIGLIVGVTSLGLLMLGLVNCIILVQRKKKPSCLQRDAKVPHVPDEKSQDAVGLEQQHLLTTAPSSSSSSLESSASAGDRRAPPGGHPQARVMAEAQGFQEARASSRISDSSHGSHGTHVNVTCIVNVCSSSDHSSQCSSQASATVGDPDAKPSASPKDEQVPFSQEECPSQSPCETTETLQSHEKPLPLGVPDMGMKPSQAGWFDQIAVKVA

SEQ ID NO: 283 - protein, 474 aa, Rattus norvegicus
MAPAALWVALVVELQLWATGHTVPAKVVLTPYKPEPGNQCQISQEYYDKKAQMCCAKCPPGQYAKHFCNKTSDTVCADCAAGMFTQVWNHLHTCLSCSSSCSDDQVETHNCTKKQNRVCACNADSYCALKLHSGNCRQCMKLSKCGPGFGVARSRTSNGNVICSACAPGTFSDTTSSTDVCRPHRICSILAIPGNASTDAVCASESPTPSAVPRTIYVSQPEPTRSQPMDQEPGPSQTPHIPVSLGSTPIIEPSITGGISLPIGLIVGLTTLGLLMLGLANCFILVQRKKKPSCLQRETMVPHLPDDKSQDAIGLEQQHLLTTAPSSSSSSLESSASAGDRRAPPGGHPQARVTAEAQGSQEACAGSRSSDSSHGSHGTHVNVTCIVNVCSSSDHSSQCSSQASTTVGDPDANPSGSPKDEQVPFSQEECPSQSQWETTETLQNHDKPFPLGVPDVGMKPNQPGWYDQIAVKVP